European Patent Application EP 4 803 537 A1, published September 9, 2026. Title: 基于Fc区的异二聚体分子及其用途. Applicant: 拓济医药（苏州）有限责任公司. The sequence listing filed with the application follows.

SEQUENCE LISTING (40 sequences)

SEQ ID NO: 1 - protein, 227 aa, synthetic construct
DKTHTCPPCPAPELLGGPSVFLFPPKPKDTLMISRTPEVTCVVVDVSHEDPEVKFNWYVDGVEVHNAKTKPREEQYNSTYRVVSVLTVLHQDWLNGKEYKCKVSNKALPAPIEKTISKAKGQPREPQVYTLPPSREEMTKNQVSLWCLVKGFYPSDIAVEWESNGQPENNYKTTPPVLDSDGSFFLYSKLTVDKSRWQQGNVFSCSVMHEALHNHYTQKSLSLSPGK

SEQ ID NO: 2 - protein, 227 aa, synthetic construct
DKTHTCPPCPAPELLGGPSVFLFPPKPKDTLMISRTPEVTCVVVDVSHEDPEVKFNWYVDGVEVHNAKTKPREEQYNSTYRVVSVLTVLHQDWLNGKEYKCKVSNKALPAPIEKTISKAKGQPREPQVYTLPPSREEMTKNQVSLWCLVKGFYPSDIAVEWESNGQPENNYKTTPPVLDSDGSFFLYSDLTVDKSRWQQGNVFSCSVMHEALHNHYTQKSLSLSPGK

SEQ ID NO: 3 - protein, 227 aa, synthetic construct
DKTHTCPPCPAPELLGGPSVFLFPPKPKDTLMISRTPEVTCVVVDVSHEDPEVKFNWYVDGVEVHNAKTKPREEQYNSTYRVVSVLTVLHQDWLNGKEYKCKVSNKALPAPIEKTISKAKGQPREPQVYTYPPSREEMTKNQVSLWCLVKGFYPSDIAVEWESNGQPENNYKTTPPVLDSDGSFFLYSKLTVDKSRWQQGNVFSCSVMHEALHNHYTQKSLSLSPGK

SEQ ID NO: 4 - protein, 227 aa, synthetic construct
DKTHTCPPCPAPELLGGPSVFLFPPKPKDTLMISRTPEVTCVVVDVSHEDPEVKFNWYVDGVEVHNAKTKPREEQYNSTYRVVSVLTVLHQDWLNGKEYKCKVSNKALPAPIEKTISKAKGQPREPQVYTYPPSREEMTKNQVSLWCLVKGFYPSDIAVEWESNGQPENNYKTTPPVLDSDGSFFLYSDLTVDKSRWQQGNVFSCSVMHEALHNHYTQKSLSLSPGK

SEQ ID NO: 5 - protein, 227 aa, synthetic construct
DKTHTCPPCPAPELLGGPSVFLFPPKPKDTLMISRTPEVTCVVVDVSHEDPEVKFNWYVDGVEVHNAKTKPREEQYNSTYRVVSVLTVLHQDWLNGKEYKCKVSNKALPAPIEKTISKAKGQPREPQVYTLPPSREEMTKNQVSLSCAVKGFYPSDIAVEWESNGQPENNYKTTPPVLDSDGSFFLVSKLTVDKSRWQQGNVFSCSVMHEALHNHYTQKSLSLSPGK

SEQ ID NO: 6 - protein, 227 aa, synthetic construct
DKTHTCPPCPAPELLGGPSVFLFPPKPKDTLMISRTPEVTCVVVDVSHEDPEVKFNWYVDGVEVHNAKTKPREEQYNSTYRVVSVLTVLHQDWLNGKEYKCKVSNKALPAPIEKTISKAKGQPREPQVYTLPPSREEMTKNQVSLSCAVKGFYPSDIAVEWESNGQPENNYKTTPPVLRSDGSFFLVSKLTVDKSRWQQGNVFSCSVMHEALHNHYTQKSLSLSPGK

SEQ ID NO: 7 - protein, 227 aa, synthetic construct
DKTHTCPPCPAPELLGGPSVFLFPPKPKDTLMISRTPEVTCVVVDVSHEDPEVKFNWYVDGVEVHNAKTKPREEQYNSTYRVVSVLTVLHQDWLNGKEYKCKVSNKALPAPIEKTISKAKGQPREPQVYTYPPSREEMTKNQVSLSCAVKGFYPSDIAVEWESNGQPENNYKTTPPVLDSDGSFFLVSKLTVDKSRWQQGNVFSCSVMHEALHNHYTQKSLSLSPGK

SEQ ID NO: 8 - protein, 227 aa, synthetic construct
DKTHTCPPCPAPELLGGPSVFLFPPKPKDTLMISRTPEVTCVVVDVSHEDPEVKFNWYVDGVEVHNAKTKPREEQYNSTYRVVSVLTVLHQDWLNGKEYKCKVSNKALPAPIEKTISKAKGQPREPQVYTYPPSREEMTKNQVSLSCAVKGFYPSDIAVEWESNGQPENNYKTTPPVLRSDGSFFLVSKLTVDKSRWQQGNVFSCSVMHEALHNHYTQKSLSLSPGK

SEQ ID NO: 9 - protein, 227 aa, synthetic construct
DKTHTCPPCPAPELLGGPSVFLFPPKPKDTLMISRTPEVTCVVVDVSHEDPEVKFNWYVDGVEVHNAKTKPREEQYNSTYRVVSVLTVLHQDWLNGKEYKCKVSNKALPAPIEKTISKAKGQPREPQVYTLPPSREEMTKNQVSLSCAVKGFYPSDIAVEWESNGQPENNYKTTPPVLKSDGSFFLVSKLTVDKSRWQQGNVFSCSVMHEALHNHYTQKSLSLSPGK

SEQ ID NO: 10 - protein, 227 aa, synthetic construct
DKTHTCPPCPAPELLGGPSVFLFPPKPKDTLMISRTPEVTCVVVDVSHEDPEVKFNWYVDGVEVHNAKTKPREEQYNSTYRVVSVLTVLHQDWLNGKEYKCKVSNKALPAPIEKTISKAKGQPREPQVYTYPPSREEMTKNQVSLSCAVKGFYPSDIAVEWESNGQPENNYKTTPPVLKSDGSFFLVSKLTVDKSRWQQGNVFSCSVMHEALHNHYTQKSLSLSPGK

SEQ ID NO: 11 - protein, 115 aa, synthetic construct [sequence omitted]

SEQ ID NO: 12 - protein, 10 aa, synthetic construct
GGGGSGGGGS

SEQ ID NO: 13 - protein, 220 aa, synthetic construct
QVQLVQSGAEVKKPGSSVKVSCKTSGYTFTDYVITWVRQAPGQGLEWMGEIYPRSDRTYYNENFKGRVTITADKSTNTAYMELSSLRSEDTAVYYCARWDNYYFDYWGQGTLVTVSSASTKGPSVFPLAPSSKSTSGGTAALGCLVKDYFPEPVTVSWNSGALTSGVHTFPAVLQSSGLYSLSSVVTVPSSSLGTQTYICNVNHKPSNTKVDKKVEPKSC

SEQ ID NO: 14 - protein, 219 aa, synthetic construct
DVVMTQSPLSLPVTLGQPASISCRSSQSLVHSNAITYLHWYQQRPGQSPRLLIYKVSNRFSGVPDRFSGSGSGTDFTLKISRVEAEDVGVYYCSQTTHVPWTFGGGTKVEIKRTVAAPSVFIFPPSDEQLKSGTASVVCLLNNFYPREAKVQWKVDNALQSGNSQESVTEQDSKDSTYSLSSTLTLSKADYEKHKVYACEVTHQGLSSPVTKSFNRGEC

SEQ ID NO: 15 - protein, 228 aa, synthetic construct
QVQLVESGGGVVQPGRSLRLSCAASGFTFSTYGMHWVRQAPGKGLEWVAVIWDDGSYKYYGDSVKGRFTISRDNSKNTLYLQMNSLRAEDTAVYYCARDGITMVRGVMKDYFDYWGQGTLVTVSSASTKGPSVFPLAPSSKSTSGGTAALGCLVKDYFPEPVTVSWNSGALTSGVHTFPAVLQSSGLYSLSSVVTVPSSSLGTQTYICNVNHKPSNTKVDKKVEPKSC

SEQ ID NO: 16 - protein, 214 aa, synthetic construct
AIQLTQSPSSLSASVGDRVTITCRASQDISSALVWYQQKPGKAPKLLIYDASSLESGVPSRFSGSESGTDFTLTISSLQPEDFATYYCQQFNSYPLTFGGGTKVEIKRTVAAPSVFIFPPSDEQLKSGTASVVCLLNNFYPREAKVQWKVDNALQSGNSQESVTEQDSKDSTYSLSSTLTLSKADYEKHKVYACEVTHQGLSSPVTKSFNRGEC

SEQ ID NO: 17 - protein, 222 aa, synthetic construct
EVQLVESGGGLVQPGGSLRLSCAASGFTFTDYTMDWVRQAPGKGLEWVADVNPNSGGSIYNQRFKGRFTLSVDRSKNTLYLQMNSLRAEDTAVYYCARNLGPSFYFDYWGQGTLVTVSSASTKGPSVFPLAPSSKSTSGGTAALGCLVKDYFPEPVTVSWNSGALTSGVHTFPAVLQSSGLYSLSSVVTVPSSSLGTQTYICNVNHKPSNTKVDKKVEPKSC

SEQ ID NO: 18 - protein, 214 aa, synthetic construct
DIQMTQSPSSLSASVGDRVTITCKASQDVSIGVAWYQQKPGKAPKLLIYSASYRYTGVPSRFSGSGSGTDFTLTISSLQPEDFATYYCQQYYIYPYTFGQGTKVEIKRTVAAPSVFIFPPSDEQLKSGTASVVCLLNNFYPREAKVQWKVDNALQSGNSQESVTEQDSKDSTYSLSSTLTLSKADYEKHKVYACEVTHQGLSSPVTKSFNRGEC

SEQ ID NO: 19 - protein, 107 aa, synthetic construct
GQPREPQVYTLPPSREEMTKNQVSLTCLVKGFYPSDIAVEWESNGQPENNYKTTPPVLDSDGSFFLYSKLTVDKSRWQQGNVFSCSVMHEALHNHYTQKSLSLSPGK

SEQ ID NO: 20 - protein, 106 aa, synthetic construct
GQPREPQVYTLPPSREEMTKNQVSLTCLVKGFYPSDIAVEWESNGQPENNYKTTPPVLDSDGSFFLYSKLTVDKSRWQQGNVFSCSVMHEALHNHYTQKSLSLSPG

SEQ ID NO: 21 - protein, 110 aa, synthetic construct
APELLGGPSVFLFPPKPKDTLMISRTPEVTCVVVDVSHEDPEVKFNWYVDGVEVHNAKTKPREEQYNSTYRVVSVLTVLHQDWLNGKEYKCKVSNKALPAPIEKTISKAK

SEQ ID NO: 22 - protein, 8 aa, synthetic construct
GGGSGGGS

SEQ ID NO: 23 - protein, 18 aa, synthetic construct
GSTSGSGKPGSGEGSTKG

SEQ ID NO: 24 - protein, 12 aa, synthetic construct
GGGSGGGSGGGS

SEQ ID NO: 25 - protein, 15 aa, synthetic construct
GGGGSGGGGSGGGGS

SEQ ID NO: 26 - protein, 16 aa, synthetic construct
GGGSGGGSGGGSGGGS

SEQ ID NO: 27 - protein, 20 aa, synthetic construct
GGGGSGGGGSGGGGSGGGGS

SEQ ID NO: 28 - protein, 20 aa, synthetic construct
GGGSGGGSGGGSGGGSGGGS

SEQ ID NO: 29 - protein, 25 aa, synthetic construct
GGGGSGGGGSGGGGSGGGGSGGGGS

SEQ ID NO: 30 - protein, 24 aa, synthetic construct
GGGSGGGSGGGSGGGSGGGSGGGS

SEQ ID NO: 31 - protein, 30 aa, synthetic construct
GGGGSGGGGSGGGGSGGGGSGGGGSGGGGS

SEQ ID NO: 32 - skipped

SEQ ID NO: 33 - protein, 5 aa, synthetic construct
DGGGS

SEQ ID NO: 34 - protein, 5 aa, synthetic construct
TGEKP

SEQ ID NO: 35 - protein, 4 aa, synthetic construct
GGRR

SEQ ID NO: 36 - protein, 14 aa, synthetic construct
EGKSSGSGSESKVD

SEQ ID NO: 37 - protein, 18 aa, synthetic construct
KESGSVSSEQLAQFRSLD

SEQ ID NO: 38 - protein, 8 aa, synthetic construct
GGRRGGGS

SEQ ID NO: 39 - protein, 9 aa, synthetic construct
LRQRDGERP

SEQ ID NO: 40 - protein, 12 aa, synthetic construct
LRQKDGGGSERP